European Patent Application EP 4 123 030 A1, published January 25, 2023. Title: DELETION MUTANTS OF E1A REGULATORY SEQUENCE. Applicant: Reid, Tony Hedjran, Farah Kumar, Shantanu University of California San Diego. The sequence listing filed with the application follows.

SEQUENCE LISTING (14 sequences)

SEQ ID NO: 1 - DNA, 58 bp, Artificial Sequence
  synthetic primer d194_243_F
aaagtgacgtttttggtgtgcgccggtgttttgggcgtaaccgagtaagatttggcca

SEQ ID NO: 2 - DNA, 58 bp, Artificial Sequence
  synthetic primer d194_243_R
tggccaaatcttactcggttacgcccaaaacaccggcgcacaccaaaaacgtcacttt

SEQ ID NO: 3 - DNA, 35 bp, Artificial Sequence
  synthetic primer dl212S
cggtgtacacaggaagtgacaatcggttttaggcg

SEQ ID NO: 4 - DNA, 35 bp, Artificial Sequence
  synthetic primer dl212 As
cgcctaaaaccgattgtcacttcctgtgtacaccg

SEQ ID NO: 5 - DNA, 34 bp, Artificial Sequence
  synthetic primer dl220S
agtgacaattttcgcgcaggcggatgttgtagta

SEQ ID NO: 6 - DNA, 34 bp, Artificial Sequence; identical to SEQ ID NO: 5
  synthetic primer dl220AS

SEQ ID NO: 7 - DNA, 41 bp, Artificial Sequence
  synthetic primer dl275S
gtaaccgagtaagatttggccatggaaaactgaataagagg

SEQ ID NO: 8 - DNA, 41 bp, Artificial Sequence
  synthetic primer dl275AS
cctcttattcagttttccatggccaaatcttactcggttac

SEQ ID NO: 9 - DNA, 30 bp, Artificial Sequence
  synthetic primer dl200S
gcgccggtgtacacagacaattttcgcgcg

SEQ ID NO: 10 - DNA, 30 bp, Artificial Sequence
  synthetic primer dl200AS
cgcgcgaaaattgtctgtgtacaccggcgc

SEQ ID NO: 11 - DNA, 34 bp, Artificial Sequence
  synthetic primer dl203S
ttcgcgcggttttaggctgtagtaaatttgggcg

SEQ ID NO: 12 - DNA, 34 bp, Artificial Sequence
  synthetic primer dl203AS
cgcccaaatttactacagcctaaaaccgcgcgaa

SEQ ID NO: 13 - DNA, 30 bp, Artificial Sequence
  synthetic primer Ad143F
ggggtaccacatgtaagcgacggatgtggc

SEQ ID NO: 14 - DNA, 27 bp, Artificial Sequence
  synthetic primer Ad552R
aaactcgagcccggtgtcggagcggct